European Patent Specification EP 3 965 793 B1, published May 1, 2024. Title: Peptides for use in therapy or prophylaxis of Herpesviridae-infections. Applicant: Eberhard Karls Universität Tübingen Medizinische Fakultät. The sequence listing filed with the application follows.

SEQUENCE LISTING (3 sequences)

SEQ ID NO: 1 - protein, 9 aa, Artificial Sequence
  Peptide derived from HD5
ATCYCRTGR

SEQ ID NO: 2 - protein, 9 aa, Artificial Sequence
  reverse sequence of SEQ ID No. 1
RGTRCYCTA

SEQ ID NO: 3 - protein, 13 aa, Artificial Sequence
  Derivative of HD5
ATCYCRTGRCATR